European Patent Specification EP 3 470 424 B1, published April 23, 2025. Title: SEQUENCE OF ANTIBODY HEAVY CHAIN CONSTANT REGION FOR ENHANCING AGONIST ANTIBODY ACTIVITY. Applicant: SHANGHAI JIAO TONG UNIVERSITY SCHOOL OF MEDICINE. Application EP17809760.6. The sequence listing filed with the application follows.

SEQUENCE LISTING (54 sequences)

SEQ ID NO: 1 - protein, 114 aa, Homo sapiens
ATTKGPSVFPLAPSSKSTSGGTAALGCLVKDYFPEPVTVSWNSGALTSGVHTFPAVLQSSGLYSLSSVVTVPSSSLGTQTYICNVNHKPSNTKVDKRVEPKSCDKTHTCPPCPA

SEQ ID NO: 2 - protein, 111 aa, Homo sapiens
ASTKGPSVFPLAPCSRSTSESTAALGCLVKDYFPEPVTVSWNSGALTSGVHTFPAVLQSSGLYSLSSVVTVPSSNFGTQTYTCNVDHKPSNTKVDKTVERKCCVECPPCPA

SEQ ID NO: 3 - protein, 161 aa, Homo sapiens
ASTKGPSVFPLAPCSRSTSGGTAALGCLVKDYFPEPVTVSWNSGALTSGVHTFPAVLQSSGLYSLSSVVTVPSSSLGTQTYTCNVNHKPSNTKVDKRVELKTPLGDTTHTCPRCPEPKSCDTPPPCPRCPEPKSCDTPPPCPRCPEPKSCDTPPPCPRCPA

SEQ ID NO: 4 - protein, 111 aa, Homo sapiens
ASTKGPSVFPLAPCSRSTSESTAALGCLVKDYFPEPVTVSWNSGALTSGVHTFPAVLQSSGLYSLSSVVTVPSSSLGTKTYTCNVDHKPSNTKVDKRVESKYGPPCPSCPA

SEQ ID NO: 5 - protein, 216 aa, Homo sapiens
PELLGGPSVFLFPPKPKDTLMISRTPEVTCVVVDVSHEDPEVKFNWYVDGVEVHNAKTKPREEQYNSTYRVVSVLTVLHQDWLNGKEYKCKVSNKALPAPIEKTISKAKGQPREPQVYTLPPSRDELTKNQVSLTCLVKGFYPSDIAVEWESNGQPENNYKTTPPVLDSDGSFFLYSKLTVDKSRWQQGNVFSCSVMHEALHNHYTQKSLSLSPGK

SEQ ID NO: 6 - protein, 215 aa, Homo sapiens
PPVAGPSVFLFPPKPKDTLMISRTPEVTCVVVDVSHEDPEVQFNWYVDGVEVHNAKTKPREEQFNSTFRVVSVLTVVHQDWLNGKEYKCKVSNKGLPAPIEKTISKTKGQPREPQVYTLPPSREEMTKNQVSLTCLVKGFYPSDIAVEWESNGQPENNYKTTPPMLDSDGSFFLYSKLTVDKSRWQQGNVFSCSVMHEALHNHYTQKSLSLSPGK

SEQ ID NO: 7 - protein, 216 aa, Homo sapiens
PELLGGPSVFLFPPKPKDTLMISRTPEVTCVVVDVSHEDPEVQFKWYVDGVEVHNAKTKPREEQYNSTFRVVSVLTVLHQDWLNGKEYKCKVSNKALPAPIEKTISKTKGQPREPQVYTLPPSREEMTKNQVSLTCLVKGFYPSDIAVEWESSGQPENNYNTTPPMLDSDGSFFLYSKLTVDKSRWQQGNIFSCSVMHEALHNRFTQKSLSLSPGK

SEQ ID NO: 8 - protein, 216 aa, Homo sapiens
PEFLGGPSVFLFPPKPKDTLMISRTPEVTCVVVDVSQEDPEVQFNWYVDGVEVHNAKTKPREEQFNSTYRVVSVLTVLHQDWLNGKEYKCKVSNKGLPSSIEKTISKAKGQPREPQVYTLPPSQEEMTKNQVSLTCLVKGFYPSDIAVEWESNGQPENNYKTTPPVLDSDGSFFLYSRLTVDKSRWQEGNVFSCSVMHEALHNHYTQKSLSLSLGK

SEQ ID NO: 9 - protein, 216 aa, Artificial sequence
  amino acid sequence for antibody IgG1 CH2-CH3 domain variant V11
PELLGDDSVFLFPPKPKDTLMISRTPEVTCVVVDVSDEDGEVKFNWYVDGVEVHNAKTKPREEQYNSTYRVVSVLTVLHQDWLNGKEYKCKVSNKALPRPIEKTISKAKGQPREPQVYTLPPSRDELTKNQVSLTCLVKGFYPSDIAVEWESNGQPENNYKTTPPVLDSDGSFFLYSKLTVDKSRWQQGNVFSCSVMHEALHNHYTQKSLSLSPGK

SEQ ID NO: 10 - protein, 216 aa, Artificial sequence
  amino acid sequence for IgG1 antibody CH2-CH3 domain variant V9
PELLGDDSVFLFPPKPKDTLMISRTPEVTCVVVDVSHEDGEVKFNWYVDGVEVHNAKTKPREEQYNSTYRVVSVLTVLHQDWLNGKEYKCKVSNKALPRPIEKTISKAKGQPREPQVYTLPPSRDELTKNQVSLTCLVKGFYPSDIAVEWESNGQPENNYKTTPPVLDSDGSFFLYSKLTVDKSRWQQGNVFSCSVMHEALHNHYTQKSLSLSPGK

SEQ ID NO: 11 - protein, 327 aa, Artificial sequence
  amino acid sequence of antibody heavy chain constant region variant JAC1
ASTKGPSVFPLAPCSRSTSESTAALGCLVKDYFPEPVTVSWNSGALTSGVHTFPAVLQSSGLYSLSSVVTVPSSNFGTQTYTCNVDHKPSNTKVDKTVERKCCVECPPCPAPELLGDDSVFLFPPKPKDTLMISRTPEVTCVVVDVSDEDGEVKFNWYVDGVEVHNAKTKPREEQYNSTYRVVSVLTVLHQDWLNGKEYKCKVSNKALPRPIEKTISKAKGQPREPQVYTLPPSRDELTKNQVSLTCLVKGFYPSDIAVEWESNGQPENNYKTTPPVLDSDGSFFLYSKLTVDKSRWQQGNVFSCSVMHEALHNHYTQKSLSLSPGK

SEQ ID NO: 12 - protein, 327 aa, Artificial sequence
  amino acid sequence of Antibody heavy chain constant region variant JAC2
ASTKGPSVFPLAPCSRSTSESTAALGCLVKDYFPEPVTVSWNSGALTSGVHTFPAVLQSSGLYSLSSVVTVPSSNFGTQTYTCNVDHKPSNTKVDKTVERKCCVECPPCPAPELLGDDSVFLFPPKPKDTLMISRTPEVTCVVVDVSHEDGEVKFNWYVDGVEVHNAKTKPREEQYNSTYRVVSVLTVLHQDWLNGKEYKCKVSNKALPRPIEKTISKAKGQPREPQVYTLPPSRDELTKNQVSLTCLVKGFYPSDIAVEWESNGQPENNYKTTPPVLDSDGSFFLYSKLTVDKSRWQQGNVFSCSVMHEALHNHYTQKSLSLSPGK

SEQ ID NO: 13 - protein, 326 aa, Artificial sequence
  amino acid sequence of Antibody heavy chain constant region variant JAC3
ASTKGPSVFPLAPCSRSTSESTAALGCLVKDYFPEPVTVSWNSGALTSGVHTFPAVLQSSGLYSLSSVVTVPSSNFGTQTYTCNVDHKPSNTKVDKTVERKCCVECPPCPAPPVAGPSVFLFPPKPKDTLMISRTPEVTCVVVDVEHEDPEVQFNWYVDGVEVHNAKTKPREEQFNSTFRVVSVLTVVHQDWLNGKEYKCKVSNKGFPAPIEKTISKTKGQPREPQVYTLPPSREEMTKNQVSLTCLVKGFYPSDIAVEWESNGQPENNYKTTPPMLDSDGSFFLYSKLTVDKSRWQQGNVFSCSVMHEALHNHYTQKSLSLSPGK

SEQ ID NO: 14 - protein, 326 aa, Artificial sequence
  amino acid sequence of Antibody heavy chain constant region variant JAC4
ASTKGPSVFPLAPCSRSTSESTAALGCLVKDYFPEPVTVSWNSGALTSGVHTFPAVLQSSGLYSLSSVVTVPSSNFGTQTYTCNVDHKPSNTKVDKTVERKCCVECPPCPAPPVAGPSVFLFPPKPKDTLMISRTPEVTCVVVDVSDEDGEVQFNWYVDGVEVHNAKTKPREEQFNSTFRVVSVLTVVHQDWLNGKEYKCKVSNKGLPAPIEKTISKTKGQPREPQVYTLPPSREEMTKNQVSLTCLVKGFYPSDIAVEWESNGQPENNYKTTPPMLDSDGSFFLYSKLTVDKSRWQQGNVFSCSVMHEALHNHYTQKSLSLSPGK

SEQ ID NO: 15 - protein, 465 aa, Artificial sequence
  amino acid sequence for the heavy chain of Human anti-murine CD40 antibody Anti-mCD40-hIgG1
MDIRLSLVFLVLFIKGVQCEVQLVESDGGLVQPGRSLKLPCAASGFTFSDYYMAWVRQAPTKGLEWVASISYDGSSTYYRDSVKGRFTISRDNAKSTLYLQMDSLRSEDTATYYCGRHSSYFDYWGQGVMVTVSSATTKGPSVFPLAPSSKSTSGGTAALGCLVKDYFPEPVTVSWNSGALTSGVHTFPAVLQSSGLYSLSSVVTVPSSSLGTQTYICNVNHKPSNTKVDKRVEPKSCDKTHTCPPCPAPELLGGPSVFLFPPKPKDTLMISRTPEVTCVVVDVSHEDPEVKFNWYVDGVEVHNAKTKPREEQYNSTYRVVSVLTVLHQDWLNGKEYKCKVSNKALPAPIEKTISKAKGQPREPQVYTLPPSRDELTKNQVSLTCLVKGFYPSDIAVEWESNGQPENNYKTTPPVLDSDGSFFLYSKLTVDKSRWQQGNVFSCSVMHEALHNHYTQKSLSLSPGK

SEQ ID NO: 16 - protein, 475 aa, Artificial sequence
  amino acid sequence for the heavy chain of Human anti-human CD40 antibody Anti-hCD40-hIgG1
MDWTWRILFLVAAATGAHSQVQLVQSGAEVKKPGASVKVSCKASGYTFTGYYMHWVRQAPGQGLEWMGWINPDSGGTNYAQKFQGRVTMTRDTSISTAYMELNRLRSDDTAVYYCARDQPLGYCTNGVCSYFDYWGQGTLVTVSSATTKGPSVFPLAPSSKSTSGGTAALGCLVKDYFPEPVTVSWNSGALTSGVHTFPAVLQSSGLYSLSSVVTVPSSSLGTQTYICNVNHKPSNTKVDKRVEPKSCDKTHTCPPCPAPELLGGPSVFLFPPKPKDTLMISRTPEVTCVVVDVSHEDPEVKFNWYVDGVEVHNAKTKPREEQYNSTYRVVSVLTVLHQDWLNGKEYKCKVSNKALPAPIEKTISKAKGQPREPQVYTLPPSRDELTKNQVSLTCLVKGFYPSDIAVEWESNGQPENNYKTTPPVLDSDGSFFLYSKLTVDKSRWQQGNVFSCSVMHEALHNHYTQKSLSLSPGK

SEQ ID NO: 17 - protein, 461 aa, Artificial sequence
  amino acid sequence for the heavy chain of Human anti-murine CD40 antibody Anti-mCD40-hIgG2
MDIRLSLVFLVLFIKGVQCEVQLVESDGGLVQPGRSLKLPCAASGFTFSDYYMAWVRQAPTKGLEWVASISYDGSSTYYRDSVKGRFTISRDNAKSTLYLQMDSLRSEDTATYYCGRHSSYFDYWGQGVMVTVSSASTKGPSVFPLAPCSRSTSESTAALGCLVKDYFPEPVTVSWNSGALTSGVHTFPAVLQSSGLYSLSSVVTVPSSNFGTQTYTCNVDHKPSNTKVDKTVERKCCVECPPCPAPPVAGPSVFLFPPKPKDTLMISRTPEVTCVVVDVSHEDPEVQFNWYVDGVEVHNAKTKPREEQFNSTFRVVSVLTVVHQDWLNGKEYKCKVSNKGLPAPIEKTISKTKGQPREPQVYTLPPSREEMTKNQVSLTCLVKGFYPSDIAVEWESNGQPENNYKTTPPMLDSDGSFFLYSKLTVDKSRWQQGNVFSCSVMHEALHNHYTQKSLSLSPGK

SEQ ID NO: 18 - protein, 471 aa, Artificial sequence
  amino acid sequence for the heavy chain of Human anti-human CD40 antibody Anti-hCD40-hIgG2
MDWTWRILFLVAAATGAHSQVQLVQSGAEVKKPGASVKVSCKASGYTFTGYYMHWVRQAPGQGLEWMGWINPDSGGTNYAQKFQGRVTMTRDTSISTAYMELNRLRSDDTAVYYCARDQPLGYCTNGVCSYFDYWGQGTLVTVSSASTKGPSVFPLAPCSRSTSESTAALGCLVKDYFPEPVTVSWNSGALTSGVHTFPAVLQSSGLYSLSSVVTVPSSNFGTQTYTCNVDHKPSNTKVDKTVERKCCVECPPCPAPPVAGPSVFLFPPKPKDTLMISRTPEVTCVVVDVSHEDPEVQFNWYVDGVEVHNAKTKPREEQFNSTFRVVSVLTVVHQDWLNGKEYKCKVSNKGLPAPIEKTISKTKGQPREPQVYTLPPSREEMTKNQVSLTCLVKGFYPSDIAVEWESNGQPENNYKTTPPMLDSDGSFFLYSKLTVDKSRWQQGNVFSCSVMHEALHNHYTQKSLSLSPGK

SEQ ID NO: 19 - protein, 512 aa, Artificial sequence
  amino acid sequence for the heavy chain of Human anti-murine CD40 antibody Anti-mCD40-hIgG3
MDIRLSLVFLVLFIKGVQCEVQLVESDGGLVQPGRSLKLPCAASGFTFSDYYMAWVRQAPTKGLEWVASISYDGSSTYYRDSVKGRFTISRDNAKSTLYLQMDSLRSEDTATYYCGRHSSYFDYWGQGVMVTVSSASTKGPSVFPLAPCSRSTSGGTAALGCLVKDYFPEPVTVSWNSGALTSGVHTFPAVLQSSGLYSLSSVVTVPSSSLGTQTYTCNVNHKPSNTKVDKRVELKTPLGDTTHTCPRCPEPKSCDTPPPCPRCPEPKSCDTPPPCPRCPEPKSCDTPPPCPRCPAPELLGGPSVFLFPPKPKDTLMISRTPEVTCVVVDVSHEDPEVQFKWYVDGVEVHNAKTKPREEQYNSTFRVVSVLTVLHQDWLNGKEYKCKVSNKALPAPIEKTISKTKGQPREPQVYTLPPSREEMTKNQVSLTCLVKGFYPSDIAVEWESSGQPENNYNTTPPMLDSDGSFFLYSKLTVDKSRWQQGNIFSCSVMHEALHNRFTQKSLSLSPGK

SEQ ID NO: 20 - protein, 522 aa, Artificial sequence
  amino acid sequence for the heavy chain of Human anti-human CD40 antibody Anti-hCD40-hIgG3
MDWTWRILFLVAAATGAHSQVQLVQSGAEVKKPGASVKVSCKASGYTFTGYYMHWVRQAPGQGLEWMGWINPDSGGTNYAQKFQGRVTMTRDTSISTAYMELNRLRSDDTAVYYCARDQPLGYCTNGVCSYFDYWGQGTLVTVSSASTKGPSVFPLAPCSRSTSGGTAALGCLVKDYFPEPVTVSWNSGALTSGVHTFPAVLQSSGLYSLSSVVTVPSSSLGTQTYTCNVNHKPSNTKVDKRVELKTPLGDTTHTCPRCPEPKSCDTPPPCPRCPEPKSCDTPPPCPRCPEPKSCDTPPPCPRCPAPELLGGPSVFLFPPKPKDTLMISRTPEVTCVVVDVSHEDPEVQFKWYVDGVEVHNAKTKPREEQYNSTFRVVSVLTVLHQDWLNGKEYKCKVSNKALPAPIEKTISKTKGQPREPQVYTLPPSREEMTKNQVSLTCLVKGFYPSDIAVEWESSGQPENNYNTTPPMLDSDGSFFLYSKLTVDKSRWQQGNIFSCSVMHEALHNRFTQKSLSLSPGK

SEQ ID NO: 21 - protein, 462 aa, Homo sapiens
  amino acid sequence for the heavy chain of Human anti-murine CD40 antibody Anti-mCD40-hIgG4
MDIRLSLVFLVLFIKGVQCEVQLVESDGGLVQPGRSLKLPCAASGFTFSDYYMAWVRQAPTKGLEWVASISYDGSSTYYRDSVKGRFTISRDNAKSTLYLQMDSLRSEDTATYYCGRHSSYFDYWGQGVMVTVSSASTKGPSVFPLAPCSRSTSESTAALGCLVKDYFPEPVTVSWNSGALTSGVHTFPAVLQSSGLYSLSSVVTVPSSSLGTKTYTCNVDHKPSNTKVDKRVESKYGPPCPSCPAPEFLGGPSVFLFPPKPKDTLMISRTPEVTCVVVDVSQEDPEVQFNWYVDGVEVHNAKTKPREEQFNSTYRVVSVLTVLHQDWLNGKEYKCKVSNKGLPSSIEKTISKAKGQPREPQVYTLPPSQEEMTKNQVSLTCLVKGFYPSDIAVEWESNGQPENNYKTTPPVLDSDGSFFLYSRLTVDKSRWQEGNVFSCSVMHEALHNHYTQKSLSLSLGK

SEQ ID NO: 22 - protein, 472 aa, Artificial sequence
  amino acid sequence for the heavy chain of Human anti-human CD40 antibody Anti-hCD40-hIgG4
MDWTWRILFLVAAATGAHSQVQLVQSGAEVKKPGASVKVSCKASGYTFTGYYMHWVRQAPGQGLEWMGWINPDSGGTNYAQKFQGRVTMTRDTSISTAYMELNRLRSDDTAVYYCARDQPLGYCTNGVCSYFDYWGQGTLVTVSSASTKGPSVFPLAPCSRSTSESTAALGCLVKDYFPEPVTVSWNSGALTSGVHTFPAVLQSSGLYSLSSVVTVPSSSLGTKTYTCNVDHKPSNTKVDKRVESKYGPPCPSCPAPEFLGGPSVFLFPPKPKDTLMISRTPEVTCVVVDVSQEDPEVQFNWYVDGVEVHNAKTKPREEQFNSTYRVVSVLTVLHQDWLNGKEYKCKVSNKGLPSSIEKTISKAKGQPREPQVYTLPPSQEEMTKNQVSLTCLVKGFYPSDIAVEWESNGQPENNYKTTPPVLDSDGSFFLYSRLTVDKSRWQEGNVFSCSVMHEALHNHYTQKSLSLSLGK

SEQ ID NO: 23 - protein, 475 aa, Artificial sequence
  amino acid sequence for the heavy chain of Human anti-human CD40 antibody Anti-hCD40-hIgG1(V9)
MDWTWRILFLVAAATGAHSQVQLVQSGAEVKKPGASVKVSCKASGYTFTGYYMHWVRQAPGQGLEWMGWINPDSGGTNYAQKFQGRVTMTRDTSISTAYMELNRLRSDDTAVYYCARDQPLGYCTNGVCSYFDYWGQGTLVTVSSATTKGPSVFPLAPSSKSTSGGTAALGCLVKDYFPEPVTVSWNSGALTSGVHTFPAVLQSSGLYSLSSVVTVPSSSLGTQTYICNVNHKPSNTKVDKRVEPKSCDKTHTCPPCPAPELLGDDSVFLFPPKPKDTLMISRTPEVTCVVVDVSHEDGEVKFNWYVDGVEVHNAKTKPREEQYNSTYRVVSVLTVLHQDWLNGKEYKCKVSNKALPRPIEKTISKAKGQPREPQVYTLPPSRDELTKNQVSLTCLVKGFYPSDIAVEWESNGQPENNYKTTPPVLDSDGSFFLYSKLTVDKSRWQQGNVFSCSVMHEALHNHYTQKSLSLSPGK

SEQ ID NO: 24 - protein, 465 aa, Artificial sequence
  amino acid sequence for the heavy chain of Human anti-murine CD40 antibody Anti-mCD40-hIgG1(V11)
MDIRLSLVFLVLFIKGVQCEVQLVESDGGLVQPGRSLKLPCAASGFTFSDYYMAWVRQAPTKGLEWVASISYDGSSTYYRDSVKGRFTISRDNAKSTLYLQMDSLRSEDTATYYCGRHSSYFDYWGQGVMVTVSSATTKGPSVFPLAPSSKSTSGGTAALGCLVKDYFPEPVTVSWNSGALTSGVHTFPAVLQSSGLYSLSSVVTVPSSSLGTQTYICNVNHKPSNTKVDKRVEPKSCDKTHTCPPCPAPELLGDDSVFLFPPKPKDTLMISRTPEVTCVVVDVSDEDGEVKFNWYVDGVEVHNAKTKPREEQYNSTYRVVSVLTVLHQDWLNGKEYKCKVSNKALPRPIEKTISKAKGQPREPQVYTLPPSRDELTKNQVSLTCLVKGFYPSDIAVEWESNGQPENNYKTTPPVLDSDGSFFLYSKLTVDKSRWQQGNVFSCSVMHEALHNHYTQKSLSLSPGK

SEQ ID NO: 25 - protein, 475 aa, Artificial sequence
  amino acid sequence for the heavy chain of Human anti-human CD40 antibody Anti-hCD40-hIgG1(V11)
MDWTWRILFLVAAATGAHSQVQLVQSGAEVKKPGASVKVSCKASGYTFTGYYMHWVRQAPGQGLEWMGWINPDSGGTNYAQKFQGRVTMTRDTSISTAYMELNRLRSDDTAVYYCARDQPLGYCTNGVCSYFDYWGQGTLVTVSSATTKGPSVFPLAPSSKSTSGGTAALGCLVKDYFPEPVTVSWNSGALTSGVHTFPAVLQSSGLYSLSSVVTVPSSSLGTQTYICNVNHKPSNTKVDKRVEPKSCDKTHTCPPCPAPELLGDDSVFLFPPKPKDTLMISRTPEVTCVVVDVSDEDGEVKFNWYVDGVEVHNAKTKPREEQYNSTYRVVSVLTVLHQDWLNGKEYKCKVSNKALPRPIEKTISKAKGQPREPQVYTLPPSRDELTKNQVSLTCLVKGFYPSDIAVEWESNGQPENNYKTTPPVLDSDGSFFLYSKLTVDKSRWQQGNVFSCSVMHEALHNHYTQKSLSLSPGK

SEQ ID NO: 26 - protein, 462 aa, Artificial sequence
  amino acid sequence for the heavy chain of Human anti-murine CD40 antibody Anti-mCD40-hIgG2(V11)
MDIRLSLVFLVLFIKGVQCEVQLVESDGGLVQPGRSLKLPCAASGFTFSDYYMAWVRQAPTKGLEWVASISYDGSSTYYRDSVKGRFTISRDNAKSTLYLQMDSLRSEDTATYYCGRHSSYFDYWGQGVMVTVSSASTKGPSVFPLAPCSRSTSESTAALGCLVKDYFPEPVTVSWNSGALTSGVHTFPAVLQSSGLYSLSSVVTVPSSNFGTQTYTCNVDHKPSNTKVDKTVERKCCVECPPCPAPELLGDDSVFLFPPKPKDTLMISRTPEVTCVVVDVSDEDGEVKFNWYVDGVEVHNAKTKPREEQYNSTYRVVSVLTVLHQDWLNGKEYKCKVSNKALPRPIEKTISKAKGQPREPQVYTLPPSRDELTKNQVSLTCLVKGFYPSDIAVEWESNGQPENNYKTTPPVLDSDGSFFLYSKLTVDKSRWQQGNVFSCSVMHEALHNHYTQKSLSLSPGK

SEQ ID NO: 27 - protein, 472 aa, Artificial sequence
  amino acid sequence for the heavy chain of Human anti-human CD40 antibody Anti-hCD40-hIgG2(V11)
MDWTWRILFLVAAATGAHSQVQLVQSGAEVKKPGASVKVSCKASGYTFTGYYMHWVRQAPGQGLEWMGWINPDSGGTNYAQKFQGRVTMTRDTSISTAYMELNRLRSDDTAVYYCARDQPLGYCTNGVCSYFDYWGQGTLVTVSSASTKGPSVFPLAPCSRSTSESTAALGCLVKDYFPEPVTVSWNSGALTSGVHTFPAVLQSSGLYSLSSVVTVPSSNFGTQTYTCNVDHKPSNTKVDKTVERKCCVECPPCPAPELLGDDSVFLFPPKPKDTLMISRTPEVTCVVVDVSDEDGEVKFNWYVDGVEVHNAKTKPREEQYNSTYRVVSVLTVLHQDWLNGKEYKCKVSNKALPRPIEKTISKAKGQPREPQVYTLPPSRDELTKNQVSLTCLVKGFYPSDIAVEWESNGQPENNYKTTPPVLDSDGSFFLYSKLTVDKSRWQQGNVFSCSVMHEALHNHYTQKSLSLSPGK

SEQ ID NO: 28 - protein, 512 aa, Artificial sequence
  amino acid sequence for the heavy chain of Human anti-murine CD40 antibody Anti-mCD40-hIgG3(V11)
MDIRLSLVFLVLFIKGVQCEVQLVESDGGLVQPGRSLKLPCAASGFTFSDYYMAWVRQAPTKGLEWVASISYDGSSTYYRDSVKGRFTISRDNAKSTLYLQMDSLRSEDTATYYCGRHSSYFDYWGQGVMVTVSSASTKGPSVFPLAPCSRSTSGGTAALGCLVKDYFPEPVTVSWNSGALTSGVHTFPAVLQSSGLYSLSSVVTVPSSSLGTQTYTCNVNHKPSNTKVDKRVELKTPLGDTTHTCPRCPEPKSCDTPPPCPRCPEPKSCDTPPPCPRCPEPKSCDTPPPCPRCPAPELLGDDSVFLFPPKPKDTLMISRTPEVTCVVVDVSDEDGEVKFNWYVDGVEVHNAKTKPREEQYNSTYRVVSVLTVLHQDWLNGKEYKCKVSNKALPRPIEKTISKAKGQPREPQVYTLPPSRDELTKNQVSLTCLVKGFYPSDIAVEWESNGQPENNYKTTPPVLDSDGSFFLYSKLTVDKSRWQQGNVFSCSVMHEALHNHYTQKSLSLSPGK

SEQ ID NO: 29 - protein, 522 aa, Artificial sequence
  amino acid sequence for the heavy chain of Human anti-human CD40 antibody Anti-hCD40-hIgG3(V11)
MDWTWRILFLVAAATGAHSQVQLVQSGAEVKKPGASVKVSCKASGYTFTGYYMHWVRQAPGQGLEWMGWINPDSGGTNYAQKFQGRVTMTRDTSISTAYMELNRLRSDDTAVYYCARDQPLGYCTNGVCSYFDYWGQGTLVTVSSASTKGPSVFPLAPCSRSTSGGTAALGCLVKDYFPEPVTVSWNSGALTSGVHTFPAVLQSSGLYSLSSVVTVPSSSLGTQTYTCNVNHKPSNTKVDKRVELKTPLGDTTHTCPRCPEPKSCDTPPPCPRCPEPKSCDTPPPCPRCPEPKSCDTPPPCPRCPAPELLGDDSVFLFPPKPKDTLMISRTPEVTCVVVDVSDEDGEVKFNWYVDGVEVHNAKTKPREEQYNSTYRVVSVLTVLHQDWLNGKEYKCKVSNKALPRPIEKTISKAKGQPREPQVYTLPPSRDELTKNQVSLTCLVKGFYPSDIAVEWESNGQPENNYKTTPPVLDSDGSFFLYSKLTVDKSRWQQGNVFSCSVMHEALHNHYTQKSLSLSPGK

SEQ ID NO: 30 - protein, 511 aa, Artificial sequence
  amino acid sequence for the heavy chain of Human anti-murine CD40 antibody Anti-mCD40-hIgG2(H3)
MDIRLSLVFLVLFIKGVQCEVQLVESDGGLVQPGRSLKLPCAASGFTFSDYYMAWVRQAPTKGLEWVASISYDGSSTYYRDSVKGRFTISRDNAKSTLYLQMDSLRSEDTATYYCGRHSSYFDYWGQGVMVTVSSASTKGPSVFPLAPCSRSTSGGTAALGCLVKDYFPEPVTVSWNSGALTSGVHTFPAVLQSSGLYSLSSVVTVPSSSLGTQTYTCNVNHKPSNTKVDKRVELKTPLGDTTHTCPRCPEPKSCDTPPPCPRCPEPKSCDTPPPCPRCPEPKSCDTPPPCPRCPAPPVAGPSVFLFPPKPKDTLMISRTPEVTCVVVDVSHEDPEVQFNWYVDGVEVHNAKTKPREEQFNSTFRVVSVLTVVHQDWLNGKEYKCKVSNKGLPAPIEKTISKTKGQPREPQVYTLPPSREEMTKNQVSLTCLVKGFYPSDIAVEWESNGQPENNYKTTPPMLDSDGSFFLYSKLTVDKSRWQQGNVFSCSVMHEALHNHYTQKSLSLSPGK

SEQ ID NO: 31 - protein, 521 aa, Artificial sequence
  amino acid sequence for the heavy chain of Human anti-human CD40 antibody Anti-hCD40-hIgG2(H3)
MDWTWRILFLVAAATGAHSQVQLVQSGAEVKKPGASVKVSCKASGYTFTGYYMHWVRQAPGQGLEWMGWINPDSGGTNYAQKFQGRVTMTRDTSISTAYMELNRLRSDDTAVYYCARDQPLGYCTNGVCSYFDYWGQGTLVTVSSASTKGPSVFPLAPCSRSTSGGTAALGCLVKDYFPEPVTVSWNSGALTSGVHTFPAVLQSSGLYSLSSVVTVPSSSLGTQTYTCNVNHKPSNTKVDKRVELKTPLGDTTHTCPRCPEPKSCDTPPPCPRCPEPKSCDTPPPCPRCPEPKSCDTPPPCPRCPAPPVAGPSVFLFPPKPKDTLMISRTPEVTCVVVDVSHEDPEVQFNWYVDGVEVHNAKTKPREEQFNSTFRVVSVLTVVHQDWLNGKEYKCKVSNKGLPAPIEKTISKTKGQPREPQVYTLPPSREEMTKNQVSLTCLVKGFYPSDIAVEWESNGQPENNYKTTPPMLDSDGSFFLYSKLTVDKSRWQQGNVFSCSVMHEALHNHYTQKSLSLSPGK

SEQ ID NO: 32 - protein, 462 aa, Artificial sequence
  amino acid sequence for the heavy chain of Human anti-murine CD40 antibody Anti-mCD40-hIgG3(H2)
MDIRLSLVFLVLFIKGVQCEVQLVESDGGLVQPGRSLKLPCAASGFTFSDYYMAWVRQAPTKGLEWVASISYDGSSTYYRDSVKGRFTISRDNAKSTLYLQMDSLRSEDTATYYCGRHSSYFDYWGQGVMVTVSSASTKGPSVFPLAPCSRSTSESTAALGCLVKDYFPEPVTVSWNSGALTSGVHTFPAVLQSSGLYSLSSVVTVPSSNFGTQTYTCNVDHKPSNTKVDKTVERKCCVECPPCPAPELLGGPSVFLFPPKPKDTLMISRTPEVTCVVVDVSHEDPEVQFKWYVDGVEVHNAKTKPREEQYNSTFRVVSVLTVLHQDWLNGKEYKCKVSNKALPAPIEKTISKTKGQPREPQVYTLPPSREEMTKNQVSLTCLVKGFYPSDIAVEWESSGQPENNYNTTPPMLDSDGSFFLYSKLTVDKSRWQQGNIFSCSVMHEALHNRFTQKSLSLSPGK

SEQ ID NO: 33 - protein, 472 aa, Artificial sequence
  amino acid sequence for the heavy chain of Human anti-human CD40 antibody Anti-hCD40-hIgG3(H2)
MDWTWRILFLVAAATGAHSQVQLVQSGAEVKKPGASVKVSCKASGYTFTGYYMHWVRQAPGQGLEWMGWINPDSGGTNYAQKFQGRVTMTRDTSISTAYMELNRLRSDDTAVYYCARDQPLGYCTNGVCSYFDYWGQGTLVTVSSASTKGPSVFPLAPCSRSTSESTAALGCLVKDYFPEPVTVSWNSGALTSGVHTFPAVLQSSGLYSLSSVVTVPSSNFGTQTYTCNVDHKPSNTKVDKTVERKCCVECPPCPAPELLGGPSVFLFPPKPKDTLMISRTPEVTCVVVDVSHEDPEVQFKWYVDGVEVHNAKTKPREEQYNSTFRVVSVLTVLHQDWLNGKEYKCKVSNKALPAPIEKTISKTKGQPREPQVYTLPPSREEMTKNQVSLTCLVKGFYPSDIAVEWESSGQPENNYNTTPPMLDSDGSFFLYSKLTVDKSRWQQGNIFSCSVMHEALHNRFTQKSLSLSPGK

SEQ ID NO: 34 - protein, 465 aa, Artificial sequence
  amino acid sequence for the heavy chain of Human anti-murine CD40 antibody Anti-mCD40-hIgG1-NA
MDIRLSLVFLVLFIKGVQCEVQLVESDGGLVQPGRSLKLPCAASGFTFSDYYMAWVRQAPTKGLEWVASISYDGSSTYYRDSVKGRFTISRDNAKSTLYLQMDSLRSEDTATYYCGRHSSYFDYWGQGVMVTVSSATTKGPSVFPLAPSSKSTSGGTAALGCLVKDYFPEPVTVSWNSGALTSGVHTFPAVLQSSGLYSLSSVVTVPSSSLGTQTYICNVNHKPSNTKVDKRVEPKSCDKTHTCPPCPAPELLGGPSVFLFPPKPKDTLMISRTPEVTCVVVDVSHEDPEVKFNWYVDGVEVHNAKTKPREEQYASTYRVVSVLTVLHQDWLNGKEYKCKVSNKALPAPIEKTISKAKGQPREPQVYTLPPSRDELTKNQVSLTCLVKGFYPSDIAVEWESNGQPENNYKTTPPVLDSDGSFFLYSKLTVDKSRWQQGNVFSCSVMHEALHNHYTQKSLSLSPGK

SEQ ID NO: 35 - protein, 475 aa, Artificial sequence
  amino acid sequence for the heavy chain of Human anti-human CD40 antibody Anti-hCD40-hIgG1-NA
MDWTWRILFLVAAATGAHSQVQLVQSGAEVKKPGASVKVSCKASGYTFTGYYMHWVRQAPGQGLEWMGWINPDSGGTNYAQKFQGRVTMTRDTSISTAYMELNRLRSDDTAVYYCARDQPLGYCTNGVCSYFDYWGQGTLVTVSSATTKGPSVFPLAPSSKSTSGGTAALGCLVKDYFPEPVTVSWNSGALTSGVHTFPAVLQSSGLYSLSSVVTVPSSSLGTQTYICNVNHKPSNTKVDKRVEPKSCDKTHTCPPCPAPELLGGPSVFLFPPKPKDTLMISRTPEVTCVVVDVSHEDPEVKFNWYVDGVEVHNAKTKPREEQYASTYRVVSVLTVLHQDWLNGKEYKCKVSNKALPAPIEKTISKAKGQPREPQVYTLPPSRDELTKNQVSLTCLVKGFYPSDIAVEWESNGQPENNYKTTPPVLDSDGSFFLYSKLTVDKSRWQQGNVFSCSVMHEALHNHYTQKSLSLSPGK

SEQ ID NO: 36 - protein, 461 aa, Artificial sequence
  amino acid sequence for the heavy chain of Human anti-murine CD40 antibody Anti-mCD40-hIgG2-NA
MDIRLSLVFLVLFIKGVQCEVQLVESDGGLVQPGRSLKLPCAASGFTFSDYYMAWVRQAPTKGLEWVASISYDGSSTYYRDSVKGRFTISRDNAKSTLYLQMDSLRSEDTATYYCGRHSSYFDYWGQGVMVTVSSASTKGPSVFPLAPCSRSTSESTAALGCLVKDYFPEPVTVSWNSGALTSGVHTFPAVLQSSGLYSLSSVVTVPSSNFGTQTYTCNVDHKPSNTKVDKTVERKCCVECPPCPAPPVAGPSVFLFPPKPKDTLMISRTPEVTCVVVDVSHEDPEVQFNWYVDGVEVHNAKTKPREEQFASTFRVVSVLTVVHQDWLNGKEYKCKVSNKGLPAPIEKTISKTKGQPREPQVYTLPPSREEMTKNQVSLTCLVKGFYPSDIAVEWESNGQPENNYKTTPPMLDSDGSFFLYSKLTVDKSRWQQGNVFSCSVMHEALHNHYTQKSLSLSPGK

SEQ ID NO: 37 - protein, 471 aa, Artificial sequence
  amino acid sequence for the heavy chain of Human anti-human CD40 antibody Anti-hCD40-hIgG2-NA
MDWTWRILFLVAAATGAHSQVQLVQSGAEVKKPGASVKVSCKASGYTFTGYYMHWVRQAPGQGLEWMGWINPDSGGTNYAQKFQGRVTMTRDTSISTAYMELNRLRSDDTAVYYCARDQPLGYCTNGVCSYFDYWGQGTLVTVSSASTKGPSVFPLAPCSRSTSESTAALGCLVKDYFPEPVTVSWNSGALTSGVHTFPAVLQSSGLYSLSSVVTVPSSNFGTQTYTCNVDHKPSNTKVDKTVERKCCVECPPCPAPPVAGPSVFLFPPKPKDTLMISRTPEVTCVVVDVSHEDPEVQFNWYVDGVEVHNAKTKPREEQFASTFRVVSVLTVVHQDWLNGKEYKCKVSNKGLPAPIEKTISKTKGQPREPQVYTLPPSREEMTKNQVSLTCLVKGFYPSDIAVEWESNGQPENNYKTTPPMLDSDGSFFLYSKLTVDKSRWQQGNVFSCSVMHEALHNHYTQKSLSLSPGK

SEQ ID NO: 38 - protein, 471 aa, Artificial sequence
  amino acid sequence for the heavy chain of Human anti-human CD40 antibody Anti-hCD40-hIgG2-SE
MDWTWRILFLVAAATGAHSQVQLVQSGAEVKKPGASVKVSCKASGYTFTGYYMHWVRQAPGQGLEWMGWINPDSGGTNYAQKFQGRVTMTRDTSISTAYMELNRLRSDDTAVYYCARDQPLGYCTNGVCSYFDYWGQGTLVTVSSASTKGPSVFPLAPCSRSTSESTAALGCLVKDYFPEPVTVSWNSGALTSGVHTFPAVLQSSGLYSLSSVVTVPSSNFGTQTYTCNVDHKPSNTKVDKTVERKCCVECPPCPAPPVAGPSVFLFPPKPKDTLMISRTPEVTCVVVDVEHEDPEVQFNWYVDGVEVHNAKTKPREEQFNSTFRVVSVLTVVHQDWLNGKEYKCKVSNKGLPAPIEKTISKTKGQPREPQVYTLPPSREEMTKNQVSLTCLVKGFYPSDIAVEWESNGQPENNYKTTPPMLDSDGSFFLYSKLTVDKSRWQQGNVFSCSVMHEALHNHYTQKSLSLSPGK

SEQ ID NO: 39 - protein, 471 aa, Artificial sequence
  amino acid sequence for the heavy chain of Human anti-human CD40 antibody Anti-hCD40-hIgG2-LF
MDWTWRILFLVAAATGAHSQVQLVQSGAEVKKPGASVKVSCKASGYTFTGYYMHWVRQAPGQGLEWMGWINPDSGGTNYAQKFQGRVTMTRDTSISTAYMELNRLRSDDTAVYYCARDQPLGYCTNGVCSYFDYWGQGTLVTVSSASTKGPSVFPLAPCSRSTSESTAALGCLVKDYFPEPVTVSWNSGALTSGVHTFPAVLQSSGLYSLSSVVTVPSSNFGTQTYTCNVDHKPSNTKVDKTVERKCCVECPPCPAPPVAGPSVFLFPPKPKDTLMISRTPEVTCVVVDVSHEDPEVQFNWYVDGVEVHNAKTKPREEQFNSTFRVVSVLTVVHQDWLNGKEYKCKVSNKGFPAPIEKTISKTKGQPREPQVYTLPPSREEMTKNQVSLTCLVKGFYPSDIAVEWESNGQPENNYKTTPPMLDSDGSFFLYSKLTVDKSRWQQGNVFSCSVMHEALHNHYTQKSLSLSPGK

SEQ ID NO: 40 - protein, 471 aa, Artificial sequence
  amino acid sequence for the heavy chain of Human anti-human CD40 antibody Anti-hCD40-hIgG2-SELF
MDWTWRILFLVAAATGAHSQVQLVQSGAEVKKPGASVKVSCKASGYTFTGYYMHWVRQAPGQGLEWMGWINPDSGGTNYAQKFQGRVTMTRDTSISTAYMELNRLRSDDTAVYYCARDQPLGYCTNGVCSYFDYWGQGTLVTVSSASTKGPSVFPLAPCSRSTSESTAALGCLVKDYFPEPVTVSWNSGALTSGVHTFPAVLQSSGLYSLSSVVTVPSSNFGTQTYTCNVDHKPSNTKVDKTVERKCCVECPPCPAPPVAGPSVFLFPPKPKDTLMISRTPEVTCVVVDVEHEDPEVQFNWYVDGVEVHNAKTKPREEQFNSTFRVVSVLTVVHQDWLNGKEYKCKVSNKGFPAPIEKTISKTKGQPREPQVYTLPPSREEMTKNQVSLTCLVKGFYPSDIAVEWESNGQPENNYKTTPPMLDSDGSFFLYSKLTVDKSRWQQGNVFSCSVMHEALHNHYTQKSLSLSPGK

SEQ ID NO: 41 - protein, 471 aa, Artificial sequence
  amino acid sequence for the heavy chain of Human anti-human CD40 antibody Anti-hCD40-hIgG2-HD
MDWTWRILFLVAAATGAHSQVQLVQSGAEVKKPGASVKVSCKASGYTFTGYYMHWVRQAPGQGLEWMGWINPDSGGTNYAQKFQGRVTMTRDTSISTAYMELNRLRSDDTAVYYCARDQPLGYCTNGVCSYFDYWGQGTLVTVSSASTKGPSVFPLAPCSRSTSESTAALGCLVKDYFPEPVTVSWNSGALTSGVHTFPAVLQSSGLYSLSSVVTVPSSNFGTQTYTCNVDHKPSNTKVDKTVERKCCVECPPCPAPPVAGPSVFLFPPKPKDTLMISRTPEVTCVVVDVSDEDPEVQFNWYVDGVEVHNAKTKPREEQFNSTFRVVSVLTVVHQDWLNGKEYKCKVSNKGLPAPIEKTISKTKGQPREPQVYTLPPSREEMTKNQVSLTCLVKGFYPSDIAVEWESNGQPENNYKTTPPMLDSDGSFFLYSKLTVDKSRWQQGNVFSCSVMHEALHNHYTQKSLSLSPGK

SEQ ID NO: 42 - protein, 471 aa, Artificial sequence
  amino acid sequence for the heavy chain of Human anti-human CD40 antibody Anti-hCD40-hIgG2-PG
MDWTWRILFLVAAATGAHSQVQLVQSGAEVKKPGASVKVSCKASGYTFTGYYMHWVRQAPGQGLEWMGWINPDSGGTNYAQKFQGRVTMTRDTSISTAYMELNRLRSDDTAVYYCARDQPLGYCTNGVCSYFDYWGQGTLVTVSSASTKGPSVFPLAPCSRSTSESTAALGCLVKDYFPEPVTVSWNSGALTSGVHTFPAVLQSSGLYSLSSVVTVPSSNFGTQTYTCNVDHKPSNTKVDKTVERKCCVECPPCPAPPVAGPSVFLFPPKPKDTLMISRTPEVTCVVVDVSHEDGEVQFNWYVDGVEVHNAKTKPREEQFNSTFRVVSVLTVVHQDWLNGKEYKCKVSNKGLPAPIEKTISKTKGQPREPQVYTLPPSREEMTKNQVSLTCLVKGFYPSDIAVEWESNGQPENNYKTTPPMLDSDGSFFLYSKLTVDKSRWQQGNVFSCSVMHEALHNHYTQKSLSLSPGK

SEQ ID NO: 43 - protein, 471 aa, Artificial sequence
  amino acid sequence for the heavy chain of Human anti-human CD40 antibody Anti-hCD40-hIgG2-HDPG
MDWTWRILFLVAAATGAHSQVQLVQSGAEVKKPGASVKVSCKASGYTFTGYYMHWVRQAPGQGLEWMGWINPDSGGTNYAQKFQGRVTMTRDTSISTAYMELNRLRSDDTAVYYCARDQPLGYCTNGVCSYFDYWGQGTLVTVSSASTKGPSVFPLAPCSRSTSESTAALGCLVKDYFPEPVTVSWNSGALTSGVHTFPAVLQSSGLYSLSSVVTVPSSNFGTQTYTCNVDHKPSNTKVDKTVERKCCVECPPCPAPPVAGPSVFLFPPKPKDTLMISRTPEVTCVVVDVSDEDGEVQFNWYVDGVEVHNAKTKPREEQFNSTFRVVSVLTVVHQDWLNGKEYKCKVSNKGLPAPIEKTISKTKGQPREPQVYTLPPSREEMTKNQVSLTCLVKGFYPSDIAVEWESNGQPENNYKTTPPMLDSDGSFFLYSKLTVDKSRWQQGNVFSCSVMHEALHNHYTQKSLSLSPGK

SEQ ID NO: 44 - protein, 466 aa, Artificial sequence
  amino acid sequence for the heavy chain of Human anti-murine DR5 antibody Anti-mDR5-hIgG2
MRLLGLLYLVTTLPGVLSQIQLQESGPGLVKPAQSLSLTCSITGFPITAGGYWWTWIRQFPGQKLEWMGYIYSSGSTNYNPSIKSRISITRDTAKNQFFLQLNSVTTEEDTAIYYCARAGTSYSGFFDSWGQGTLVTVSSASTKGPSVFPLAPCSRSTSESTAALGCLVKDYFPEPVTVSWNSGALTSGVHTFPAVLQSSGLYSLSSVVTVPSSNFGTQTYTCNVDHKPSNTKVDKTVERKCCVECPPCPAPPVAGPSVFLFPPKPKDTLMISRTPEVTCVVVDVSHEDPEVQFNWYVDGVEVHNAKTKPREEQFNSTFRVVSVLTVVHQDWLNGKEYKCKVSNKGLPAPIEKTISKTKGQPREPQVYTLPPSREEMTKNQVSLTCLVKGFYPSDIAVEWESNGQPENNYKTTPPMLDSDGSFFLYSKLTVDKSRWQQGNVFSCSVMHEALHNHYTQKSLSLSPGK

SEQ ID NO: 45 - protein, 470 aa, Artificial sequence
  amino acid sequence for the heavy chain of Human anti-murine DR5 antibody Anti-mDR5-hIgG1(V11)
MRLLGLLYLVTTLPGVLSQIQLQESGPGLVKPAQSLSLTCSITGFPITAGGYWWTWIRQFPGQKLEWMGYIYSSGSTNYNPSIKSRISITRDTAKNQFFLQLNSVTTEEDTAIYYCARAGTSYSGFFDSWGQGTLVTVSSATTKGPSVFPLAPSSKSTSGGTAALGCLVKDYFPEPVTVSWNSGALTSGVHTFPAVLQSSGLYSLSSVVTVPSSSLGTQTYICNVNHKPSNTKVDKRVEPKSCDKTHTCPPCPAPELLGDDSVFLFPPKPKDTLMISRTPEVTCVVVDVSDEDGEVKFNWYVDGVEVHNAKTKPREEQYNSTYRVVSVLTVLHQDWLNGKEYKCKVSNKALPRPIEKTISKAKGQPREPQVYTLPPSRDELTKNQVSLTCLVKGFYPSDIAVEWESNGQPENNYKTTPPVLDSDGSFFLYSKLTVDKSRWQQGNVFSCSVMHEALHNHYTQKSLSLSPGK

SEQ ID NO: 46 - protein, 467 aa, Artificial sequence
  amino acid sequence for the heavy chain of Human anti-murine DR5 antibody Anti-mDR5-IgG2(V11)
MRLLGLLYLVTTLPGVLSQIQLQESGPGLVKPAQSLSLTCSITGFPITAGGYWWTWIRQFPGQKLEWMGYIYSSGSTNYNPSIKSRISITRDTAKNQFFLQLNSVTTEEDTAIYYCARAGTSYSGFFDSWGQGTLVTVSSASTKGPSVFPLAPCSRSTSESTAALGCLVKDYFPEPVTVSWNSGALTSGVHTFPAVLQSSGLYSLSSVVTVPSSNFGTQTYTCNVDHKPSNTKVDKTVERKCCVECPPCPAPELLGDDSVFLFPPKPKDTLMISRTPEVTCVVVDVSDEDGEVKFNWYVDGVEVHNAKTKPREEQYNSTYRVVSVLTVLHQDWLNGKEYKCKVSNKALPRPIEKTISKAKGQPREPQVYTLPPSRDELTKNQVSLTCLVKGFYPSDIAVEWESNGQPENNYKTTPPVLDSDGSFFLYSKLTVDKSRWQQGNVFSCSVMHEALHNHYTQKSLSLSPGK

SEQ ID NO: 47 - protein, 234 aa, Artificial sequence
  amino acid sequence for the light chain of Human anti-human CD40 antibody
MRLPAQLLGLLLLWFPGSRCDIQMTQSPSSVSASVGDRVTITCRASQGIYSWLAWYQQKPGKAPNLLIYTASTLQSGVPSRFSGSGSGTDFTLTISSLQPEDFATYYCQQANIFPLTFGGGTKVEIKRTVAAPSVFIFPPSDEQLKSGTASVVCLLNNFYPREAKVQWKVDNALQSGNSQESVTEQDSKDSTYSLSSTLTLSKADYEKHKVYACEVTHQGLSSPVTKSFNRGEC

SEQ ID NO: 48 - protein, 233 aa, Artificial sequence
  amino acid sequence for the light chain of Human anti-murine CD40 antibody
METDRLLLWVLLLWVPGSTGDTVLTQSPALAVSPGERVTISCRASDSVSTLMHWYQQKPGQQPKLLIYLASHLESGVPARFSGSGSGTDFTLTIDPVEADDTATYYCQQSWNDPWTFGGGTKLELKRTVAAPSVFIFPPSDEQLKSGTASVVCLLNNFYPREAKVQWKVDNALQSGNSQESVTEQDSKDSTYSLSSTLTLSKADYEKHKVYACEVTHQGLSSPVTKSFNRGEC

SEQ ID NO: 49 - protein, 236 aa, Artificial sequence
  amino acid sequence for the light chain of Human anti-murine DR5
MAMKVPAQALVILLLWVSGATCDIQVTQSPSLLSASFGDKVTINCLVTQDITYYLSWYQQKSGQPPTLLIYNGNSLQSGVPSRFSGQYSGRTFTLSLSSLEPEDAGTYYCLQHYSVPFTFGGGTRLEIKRTVAAPSVFIFPPSDEQLKSGTASVVCLLNNFYPREAKVQWKVDNALQSGNSQESVTEQDSKDSTYSLSSTLTLSKADYEKHKVYACEVTHQGLSSPVTKSFNRGEC

SEQ ID NO: 50 - protein, 464 aa, Artificial sequence
  amino acid sequence for the heavy chain of Human anti-murine CD40 antibody Anti-mCD40-hIgG1-SDIE
MDIRLSLVFLVLFIKGVQCEVQLVESDGGLVQPGRSLKLPCAASGFTFSDYYMAWVRQAPTKGLEWVASISYDGSSTYYRDSVKGRFTISRDNAKSTLYLQMDSLRSEDTATYYCGRHSSYFDYWGQGVMVTVSSASTKGPSVFPLAPSSKSTSGGTAALGCLVKDYFPEPVTVSWNSGALTSGVHTFPAVLQSSGLYSLSSVVTVPSSSLGTQTYICNVNHKPSNTKVDKRVEPKSCDKTHTCPPCPAPELLGGPDVFLFPPKPKDTLMISRTPEVTCVVVDVSHEDPEVKFNWYVDGVEVHNAKTKPREEQYNSTYRVVSVLTVLHQDWLNGKEYKCKVSNKALPAPEEKTISKAKGQPREPQVYTLPPSRDELTKNQVSLTCLVKGFYPSDIAVEWESNGQPENNYKTTPPVLDSDGSFFLYSKLTVDKSRWQQGNVFSCSVMHEALHNHYTQKSLLPVSG

SEQ ID NO: 51 - protein, 461 aa, Artificial sequence
  amino acid sequence for the heavy chain of Human anti-murine CD40 antibody Anti-mCD40-hIgG2-SDIE
MDIRLSLVFLVLFIKGVQCEVQLVESDGGLVQPGRSLKLPCAASGFTFSDYYMAWVRQAPTKGLEWVASISYDGSSTYYRDSVKGRFTISRDNAKSTLYLQMDSLRSEDTATYYCGRHSSYFDYWGQGVMVTVSSASTKGPSVFPLAPCSRSTSESTAALGCLVKDYFPEPVTVSWNSGALTSGVHTFPAVLQSSGLYSLSSVVTVPSSNFGTQTYTCNVDHKPSNTKVDKTVERKCCVECPPCPAPELLGGPDVFLFPPKPKDTLMISRTPEVTCVVVDVSHEDPEVKFNWYVDGVEVHNAKTKPREEQYNSTYRVVSVLTVLHQDWLNGKEYKCKVSNKALPAPEEKTISKAKGQPREPQVYTLPPSRDELTKNQVSLTCLVKGFYPSDIAVEWESNGQPENNYKTTPPVLDSDGSFFLYSKLTVDKSRWQQGNVFSCSVMHEALHNHYTQKSLLPVSG

SEQ ID NO: 52 - protein, 462 aa, Artificial sequence
  amino acid sequence for the heavy chain of Human anti-murine CD40 antibody Anti-mCD40-hIgG2-GASDALIE
MDIRLSLVFLVLFIKGVQCEVQLVESDGGLVQPGRSLKLPCAASGFTFSDYYMAWVRQAPTKGLEWVASISYDGSSTYYRDSVKGRFTISRDNAKSTLYLQMDSLRSEDTATYYCGRHSSYFDYWGQGVMVTVSSASTKGPSVFPLAPCSRSTSESTAALGCLVKDYFPEPVTVSWNSGALTSGVHTFPAVLQSSGLYSLSSVVTVPSSNFGTQTYTCNVDHKPSNTKVDKTVERKCCVECPPCPAPELLAGPDVFLFPPKPKDTLMISRTPEVTCVVVDVSHEDPEVKFNWYVDGVEVHNAKTKPREEQYNSTYRVVSVLTVLHQDWLNGKEYKCKVSNKALPLPEEKTISKAKGQPREPQVYTLPPSRDELTKNQVSLTCLVKGFYPSDIAVEWESNGQPENNYKTTPPVLDSDGSFFLYSKLTVDKSRWQQGNVFSCSVMHEALHNHYTQKSLSLSPGK

SEQ ID NO: 53 - protein, 462 aa, Artificial sequence
  amino acid sequence for the heavy chain of Human anti-murine CD40 antibody Anti-mCD40-hIgG1-H1
MDIRLSLVFLVLFIKGVQCEVQLVESDGGLVQPGRSLKLPCAASGFTFSDYYMAWVRQAPTKGLEWVASISYDGSSTYYRDSVKGRFTISRDNAKSTLYLQMDSLRSEDTATYYCGRHSSYFDYWGQGVMVTVSSASTKGPSVFPLAPCSRSTSESTAALGCLVKDYFPEPVTVSWNSGALTSGVHTFPAVLQSSGLYSLSSVVTVPSSNFGTQTYTCNVDHKPSNTKVDKTVERKCCVECPPCPAPELLGGPSVFLFPPKPKDTLMISRTPEVTCVVVDVSHEDPEVKFNWYVDGVEVHNAKTKPREEQYNSTYRVVSVLTVLHQDWLNGKEYKCKVSNKALPAPIEKTISKAKGQPREPQVYTLPPSRDELTKNQVSLTCLVKGFYPSDIAVEWESNGQPENNYKTTPPVLDSDGSFFLYSKLTVDKSRWQQGNVFSCSVMHEALHNHYTQKSLSLSPGK

SEQ ID NO: 54 - protein, 470 aa, Artificial sequence
  amino acid sequence for the heavy chain of Human anti-murine DR5 antibody Anti-mDR5-hIgG1-GASDALIE
MRLLGLLYLVTTLPGVLSQIQLQESGPGLVKPAQSLSLTCSITGFPITAGGYWWTWIRQFPGQKLEWMGYIYSSGSTNYNPSIKSRISITRDTAKNQFFLQLNSVTTEEDTAIYYCARAGTSYSGFFDSWGQGTLVTVSSATTKGPSVFPLAPSSKSTSGGTAALGCLVKDYFPEPVTVSWNSGALTSGVHTFPAVLQSSGLYSLSSVVTVPSSSLGTQTYICNVNHKPSNTKVDKRVEPKSCDKTHTCPPCPAPELLAGPDVFLFPPKPKDTLMISRTPEVTCVVVDVSHEDPEVKFNWYVDGVEVHNAKTKPREEQYNSTYRVVSVLTVLHQDWLNGKEYKCKVSNKALPLPEEKTISKAKGQPREPQVYTLPPSRDELTKNQVSLTCLVKGFYPSDIAVEWESNGQPENNYKTTPPVLDSDGSFFLYSKLTVDKSRWQQGNVFSCSVMHEALHNHYTQKSLSLSPGK